European Patent Application EP 4 737 560 A1, published May 6, 2026. Title: MESENCHYMAL STEM CELL-DERIVED EXTRACELLULAR VESICLES AND USE THEREOF. Applicant: 코아스템켐온 주식회사. The sequence listing filed with the application follows.

SEQUENCE LISTING (40 sequences)

SEQ ID NO: 1 - DNA, 22 bp, synthetic construct
  source 1..22: mol_type = other DNA
  misc_feature 1..22: note = TGF-beta1 F
tacctgaacccgtgttgctctc

SEQ ID NO: 2 - DNA, 21 bp, synthetic construct
  source 1..21: mol_type = other DNA
  misc_feature 1..21: note = TGF-beta1 R
gttgctgaggtatcgccagga

SEQ ID NO: 3 - DNA, 22 bp, synthetic construct
  source 1..22: mol_type = other DNA
  misc_feature 1..22: note = Vimentin F
aggcaaagcaggagtccactga

SEQ ID NO: 4 - DNA, 22 bp, synthetic construct
  source 1..22: mol_type = other DNA
  misc_feature 1..22: note = Vimentin R
atctggcgttccagggactcat

SEQ ID NO: 5 - DNA, 22 bp, synthetic construct
  source 1..22: mol_type = other DNA
  misc_feature 1..22: note = CTGF F
cttgcgaagctgacctggaaga

SEQ ID NO: 6 - DNA, 22 bp, synthetic construct
  source 1..22: mol_type = other DNA
  misc_feature 1..22: note = CTGF R
ccgtcggtacatactccacaga

SEQ ID NO: 7 - DNA, 20 bp, synthetic construct
  source 1..20: mol_type = other DNA
  misc_feature 1..20: note = COL3A1 F
gaccctaaccaaggatgcaa

SEQ ID NO: 8 - DNA, 20 bp, synthetic construct
  source 1..20: mol_type = other DNA
  misc_feature 1..20: note = COL3A1 R
ggaagttcaggattgccgta

SEQ ID NO: 9 - DNA, 23 bp, synthetic construct
  source 1..23: mol_type = other DNA
  misc_feature 1..23: note = E-cadherin F
gcctcctgaaaagagagtggaag

SEQ ID NO: 10 - DNA, 22 bp, synthetic construct
  source 1..22: mol_type = other DNA
  misc_feature 1..22: note = E-cadherin R
tggcagtgtctctccaaatccg

SEQ ID NO: 11 - RNA, 22 nt, synthetic construct
  source 1..22: mol_type = other RNA
  misc_feature 1..22: note = GAPDH F
gtctcctctgacttcaacagcg

SEQ ID NO: 12 - DNA, 22 bp, synthetic construct
  source 1..22: mol_type = other DNA
  misc_feature 1..22: note = GAPDH R
accaccctgttgctgtagccaa

SEQ ID NO: 13 - DNA, 19 bp, synthetic construct
  source 1..19: mol_type = other DNA
  misc_feature 1..19: note = mCOL1A1 F
tcctccagggatccaacga

SEQ ID NO: 14 - DNA, 17 bp, synthetic construct
  source 1..17: mol_type = other DNA
  misc_feature 1..17: note = mCOL1A1 R
ggcaggcgggaggtctt

SEQ ID NO: 15 - DNA, 20 bp, synthetic construct
  source 1..20: mol_type = other DNA
  misc_feature 1..20: note = mCOL3A1 F
gtgaaactggtgaacgtggc

SEQ ID NO: 16 - DNA, 20 bp, synthetic construct
  source 1..20: mol_type = other DNA
  misc_feature 1..20: note = mCOL3A1 R
ataggacctggatgcccact

SEQ ID NO: 17 - DNA, 19 bp, synthetic construct
  source 1..19: mol_type = other DNA
  misc_feature 1..19: note = mCTGF F
gggcctcttctgcgatttc

SEQ ID NO: 18 - DNA, 21 bp, synthetic construct
  source 1..21: mol_type = other DNA
  misc_feature 1..21: note = mCTGF R
atccaggcaagtgcattggta

SEQ ID NO: 19 - DNA, 21 bp, synthetic construct
  source 1..21: mol_type = other DNA
  misc_feature 1..21: note = mElastin F
ttgctgatcctcttgctcaac

SEQ ID NO: 20 - DNA, 22 bp, synthetic construct
  source 1..22: mol_type = other DNA
  misc_feature 1..22: note = mElastin R
gcccctggataatagactccac

SEQ ID NO: 21 - DNA, 19 bp, synthetic construct
  source 1..19: mol_type = other DNA
  misc_feature 1..19: note = mRPL13A F
ccctcaccctatgacaaga

SEQ ID NO: 22 - DNA, 20 bp, synthetic construct
  source 1..20: mol_type = other DNA
  misc_feature 1..20: note = mRPL13A R
ccttttccttccgtttctcc

SEQ ID NO: 23 - DNA, 21 bp, synthetic construct
  source 1..21: mol_type = other DNA
  misc_feature 1..21: note = mTimp1 F
gcaactcggacctggtcataa

SEQ ID NO: 24 - DNA, 19 bp, synthetic construct
  source 1..19: mol_type = other DNA
  misc_feature 1..19: note = mTimp1 R
cggcccgtgatgagaaact

SEQ ID NO: 25 - DNA, 21 bp, synthetic construct
  source 1..21: mol_type = other DNA
  misc_feature 1..21: note = malpha-SMA F
gtcccagacatcagggagtaa

SEQ ID NO: 26 - DNA, 21 bp, synthetic construct
  source 1..21: mol_type = other DNA
  misc_feature 1..21: note = malpha-SMA R
tcggatacttcagcgtcagga

SEQ ID NO: 27 - DNA, 20 bp, synthetic construct
  source 1..20: mol_type = other DNA
  misc_feature 1..20: note = mFibronectin F
tgacgctggctttaagctca

SEQ ID NO: 28 - RNA, 20 nt, synthetic construct
  source 1..20: mol_type = other RNA
  misc_feature 1..20: note = mFibronectin R
tcatccgctggccattttct

SEQ ID NO: 29 - DNA, 22 bp, synthetic construct
  source 1..22: mol_type = other DNA
  misc_feature 1..22: note = Fibronectin F
acaacaccgaggtgactgagac

SEQ ID NO: 30 - DNA, 22 bp, synthetic construct
  source 1..22: mol_type = other DNA
  misc_feature 1..22: note = Fibronectin R
ggacacaacgatgcttcctgag

SEQ ID NO: 31 - DNA, 21 bp, synthetic construct
  source 1..21: mol_type = other DNA
  misc_feature 1..21: note = alpha-SMA F
ctttctacaatgagcttcgtg

SEQ ID NO: 32 - DNA, 20 bp, synthetic construct
  source 1..20: mol_type = other DNA
  misc_feature 1..20: note = alpha-SMA R
atttgagtcattttctcccg

SEQ ID NO: 33 - DNA, 25 bp, synthetic construct
  source 1..25: mol_type = other DNA
  misc_feature 1..25: note = beta-actin F
tggaatcctgtggcatccatgaaac

SEQ ID NO: 34 - DNA, 25 bp, synthetic construct
  source 1..25: mol_type = other DNA
  misc_feature 1..25: note = beta-actin R
taaaacgcagctcagtaacagtccg

SEQ ID NO: 35 - RNA, 22 nt, synthetic construct
  source 1..22: mol_type = other RNA
  misc_feature 1..22: note = miR-148a-3p
acaaagttctgtagtgcactga

SEQ ID NO: 36 - RNA, 22 nt, synthetic construct
  source 1..22: mol_type = other RNA
  misc_feature 1..22: note = Let-7a-5p
aactatacaacctactacctca

SEQ ID NO: 37 - RNA, 22 nt, synthetic construct
  source 1..22: mol_type = other RNA
  misc_feature 1..22: note = Let-7b-5p
aaccacacaacctactacctca

SEQ ID NO: 38 - DNA, 22 bp, synthetic construct
  source 1..22: mol_type = other DNA
  misc_feature 1..22: note = miR-100-5p
cacaagttcggatctacgggtt

SEQ ID NO: 39 - RNA, 21 nt, synthetic construct
  source 1..21: mol_type = other RNA
  misc_feature 1..21: note = miR-143-3p
gagctacagtgcttcatctca

SEQ ID NO: 40 - RNA, 22 nt, synthetic construct
  source 1..22: mol_type = other RNA
  misc_feature 1..22: note = Let-7f-5p
aactatacaatctactacctca